European Patent Specification EP 4 039 819 B1, published August 14, 2024. Title: METHOD FOR ASSESSING RISK OF CUTANEOUS ADVERSE DRUG REACTIONS CAUSED BY EPIDERMAL GROWTH FACTOR RECEPTOR INHIBITOR, DETECTION KIT THEREOF, AND USE THEREOF. Applicant: Chang Gung Memorial Hospital, Linkou. The sequence listing filed with the application follows.

SEQUENCE LISTING (8 sequences)

SEQ ID NO: 1 - DNA, 18 bp, Artificial Sequence
  Forward primer 1
cgcttcattgcagtgggc

SEQ ID NO: 2 - DNA, 24 bp, Artificial Sequence
  Reverse prmer 1
tggtcttgaagatctgtgtgttcc

SEQ ID NO: 3 - DNA, 14 bp, Artificial Sequence
  Probe 1
agagaggagccgcg

SEQ ID NO: 4 - DNA, 13 bp, Artificial Sequence
  Probe 2
gacggagccccgg

SEQ ID NO: 5 - DNA, 22 bp, Artificial Sequence
  Foward Primer 2
acacttggcagacgatgtatgg

SEQ ID NO: 6 - DNA, 19 bp, Artificial Sequence
  Reverse Primer 2
ggtccaggagctcaggtcc

SEQ ID NO: 7 - DNA, 15 bp, Artificial Sequence
  Probe 3
cggcaaggattacat

SEQ ID NO: 8 - DNA, 16 bp, Artificial Sequence
  Probe 4
acggcaaagattacat